European Patent Specification EP 3 557 982 B1, published April 29, 2026. Title: PROLIFIC FLOWERING WATERMELON. Applicant: Syngenta Participations AG Brusca, James  P Kinkade, Matt Danan, Sarah. The sequence listing filed with the application follows.

SEQUENCE LISTING (9 sequences)

SEQ ID NO: 1 - DNA, 20 bp, Artificial Sequence
  Primer
cgttgagacgttcgctgttc

SEQ ID NO: 2 - DNA, 21 bp, Artificial Sequence
  Primer
gacggagacccatgataagga

SEQ ID NO: 3 - DNA, 201 bp, Citrullus lanatus
gctcgtagccgtcgttggtctctacgccatgtccgctcgccgccacgtcgagatgccrtcgttttcgtcgtcgttgagacgttcgctgttcgtcccttttggttcctcgaccaccagcgtctccttatcatgggtctccgtcgtttgcagtcgccgccggttctcatcctcacacctgctgccgtcaaccaacgaccctcc

SEQ ID NO: 4 - DNA, 22 bp, Artificial Sequence
  Primer
ggtcggcaatgactagacgaat

SEQ ID NO: 5 - DNA, 20 bp, Artificial Sequence
  Primer
tcctccatcgctccaaacct

SEQ ID NO: 6 - DNA, 201 bp, Citrullus lanatus
cgttaaaataaaaaaataaaaaaaataaaaaaagcctttagcagcgacaaatgatagagggtggtcggcaatgactagacgaatggaagcaccatgagagaaaaggaggtttggagcgatggaggagatcagagatgaggagagggatcaaatttggggaccacgaactcgtggaccccctccmcgagttacctgctaagt

SEQ ID NO: 7 - DNA, 24 bp, Artificial Sequence
  Primer
tcgacaaatggagaaggttcaact

SEQ ID NO: 8 - DNA, 21 bp, Artificial Sequence
  Primer
acctttgtgtccttcccagaa

SEQ ID NO: 9 - DNA, 201 bp, Citrullus lanatus
gattgataaaatccacaacaaattcgacaaatggagaaggttcaacttatctagaagtgggagggccactttatataagtctattctttccaatcttccaccatattatatgtctctatttctaatgcctgaaaaggttgtctctatattgaaaaagaataatgcggaacttcttctgggaaggacacaaaggtagcataa